European Patent Application EP 4 371 569 A1, published May 22, 2024. Title: VLPs AGAINST ACUTE MYELOID LEUKAEMIA. Applicant: Universidad del País Vasco. The sequence listing filed with the application follows.

SEQUENCE LISTING (12 sequences)

SEQ ID NO: 1 - protein, 9 aa, Synthetic construct
  REGION 1..9: note = AVEEVSLRK peptide
AVEEVSLRK

SEQ ID NO: 2 - protein, 9 aa, Synthetic construct
  REGION 1..9: note = RMFPNAPYL peptide
RMFPNAPYL

SEQ ID NO: 3 - protein, 20 aa, Synthetic construct
  REGION 1..20: note = GWVKPIIIGHHAYGDQYRAT peptide
GWVKPIIIGHHAYGDQYRAT

SEQ ID NO: 4 - protein, 10 aa, Synthetic construct
  REGION 1..10: note = YVDFREYEYY peptide
YVDFREYEYY

SEQ ID NO: 5-7 - skipped (3 entries)

SEQ ID NO: 8 - protein, 15 aa, Synthetic construct
  REGION 1..15: note = BAP
GLNDIFEAQKIEWHE

SEQ ID NO: 9 - DNA, 36 bp
ccggaattcatgctcgctgtaaataatgtaaatatg

SEQ ID NO: 10 - DNA, 70 bp, Synthetic construct
  source 1..70: mol_type = other DNA; note = Primer
ttaaaagcggccgcctattttcttaaagatacttcttcaacagcagatagataaaaatttgagaaggtag

SEQ ID NO: 11 - protein, 868 aa, Triatoma virus
  REGION 1..868: note = TrV structural proteins
LAVNNVNMKQMNVNSSQDTTFEQRSQEKVQAGEINESIEFRNQITTFVHDNPIITEQLIGDSPQPSGDVRSVSDARTHSIIDFLERPQFIGSFLWNTSDIENKEIFSLKLPDALMSPMIREKLSGFTSFSASTVFHIQVNAHPFQCGRLVLAAVPVPDILPLHRLNMLSFDVSNVITLPHVQLDISKETEVLLKIPYVSPFVQYDLVTKFTPWAAFLAHVYAPLNTPSAASLQVNVFAHFEDIKLGFPTSAIVAQAGKEQLGPISGLTNTVTGVVGGVADAVKGFFPSIGKYADPLVGIGNGLTGLLSALGFSKPLTTIPPTIVVQRPSQYFNNADGVDQGLPLSLKYGNEVILKTPFAGTSSDEVALEYVLKIPNYFSRFKYSSTSLPKQVLWYSPVHPQIIRNHVTVVDAPGQPTLLAYATGFFKYWRGGLVYTFRFVKTNYHSGRVQITFHPFVGYDDVMDSDGKIVRDEYVYRVVVDLRDQTEATLVVPFTSLTPYKVCADVFNSANRPKYNYEPRDFKVYDNTTDQFFTGTLCVSALTPLVSSSAVVSSTIDVLVEVKASDDFEVAVPNTPLWLPVDSLTERPSLDGVPIAQVGFASAGTRDIRSSYVEGKFIPQDITGMSRNHELDEQPSQECIGERILSFSELIKRNSWRYVSDEKSLIYPAYAFDNPAAMYTAADKLPVWTLTPRSGFPTLLTSIGAMYAFYRGGIRLKIVPGVADQPKPLVEVALFTMQDQGYIIKANDYSTDFCSSNIYENFVTKGIAEVQTPYYSRVNTSVVSAPVLYNAGNISPLMPNVMYKITSNSSNILLGHSAADDFRFGFLLGAPLAISATALRDNFTGSSATVSLPTFSNFYLSSTSESTT

SEQ ID NO: 12 - protein, 273 aa, Synthetic construct
  REGION 1..273: note = vaccine against AML-NPMc+
VGFASAGTRDIRSSYVEGKFIPQDITGMSRNHELDEQPSQECIGERILSFSELIKRNSWRYVSDEKSLIYPAYAFDNPAAMYTAADKLPVWTLTPRSGFPTLLTSIGAMYAFYRGGIRLKIVPGVADQPKPLVEVALFTMQDQGYIIKANDYSTDFCSSNIYENFVTKGIAEVQTPYYSRVNTSVVSAPVLYNAGNISPLMPNVMYKITSNSSNILLGHSAADDFRFGFLLGAPLAISATALRDNFTGSSATVSLPTFSNFYLSAVEEVSLRK